European Patent Application EP 4 349 857 A1, published April 10, 2024. Title: MONOBODY BASED CHIMERIC ANTIGEN RECEPTOR AND IMMUNE CELL COMPRISING THEREOF. Applicant: Vaxcell-Bio. The sequence listing filed with the application follows.

SEQUENCE LISTING (16 sequences)

SEQ ID NO: 1 - DNA, 63 bp, Artificial Sequence
  CD8alpha signal sequence nucleotide
atggccctgcctgtgacagctttgctgctgcctctggctctgctgctgcatgctgctagacct

SEQ ID NO: 2 - DNA, 270 bp, Artificial Sequence
  E1 monomer nucleotide
gtttctgatgttccgagggacctggaagttgttgctgcgacccccaccagcctactgatcagctggtattatccgttttgtgcgttttattacaggatcacttacggagaaacaggaggaaatagccctgtccaggagttcactgtgcctcgtccgtctgacactgctaccatcagcggccttaaacctggagttgattataccatcactgtgtatgctgtcacgtgtctgggctcgtattctcgcccaatttccattaattaccgaaca

SEQ ID NO: 3 - DNA, 207 bp, Artificial Sequence
  CD8alpha H&TM nucleotide
accaccacaccagctccacggcctccaacaccagcacctacaattgcctctcagcccctgtctctgaggccagaagcttgtagacctgctgcaggcggagccgtgcataccagaggactggatttcgcctgcgacatctacatttgggcccctctggctggaacatgtggcgtcctgctgctgtctctcgtgatcaccctgtactgc

SEQ ID NO: 4 - DNA, 123 bp, Artificial Sequence
  CD28 nucleotide
agaagcaagagaagccggctgctgcacagcgactacatgaacatgacccctagacggcccggacctaccagaaagcactaccagccttacgctcctcctcgggactttgccgcctatagatcc

SEQ ID NO: 5 - DNA, 126 bp, Artificial Sequence
  4-1BB nucleotide
aagcggggcagaaagaagctgctgtacatcttcaagcagcccttcatgcggcccgtgcagaccacacaagaggaagatggctgctcctgcagattccccgaggaagaagaaggcggctgcgagctg

SEQ ID NO: 6 - DNA, 339 bp, Artificial Sequence
  CD3zeta nucleotide
agagtgaagttctctagatctgccgacgctcctgcctaccagcagggacagaatcagctgtacaacgagctgaatctggggcgcagagaagagtacgacgtgctggataagagaagaggcagagatcccgagatgggcggcaagccccagagaagaaagaatccccaagagggcctgtataatgagctgcagaaagacaagatggccgaggcctacagcgagatcggaatgaagggcgaacgcagaagaggaaagggccacgacggactgtatcagggcctgagcacagccaccaaggatacctatgatgccctgcacatgcaggccctgccacctagg

SEQ ID NO: 7 - protein, 21 aa, Artificial Sequence
  CD8alpha signal sequence amino acid
MALPVTALLLPLALLLHAARP

SEQ ID NO: 8 - protein, 90 aa, Artificial Sequence
  E1 monomer amino acid
VSDVPRDLEVVAATPTSLLISWYYPFCAFYYRITYGETGGNSPVQEFTVPRPSDTATISGLKPGVDYTITVYAVTCLGSYSRPISINYRT

SEQ ID NO: 9 - protein, 69 aa, Artificial Sequence
  CD8alpha H&TM amino acid
TTTPAPRPPTPAPTIASQPLSLRPEACRPAAGGAVHTRGLDFACDIYIWAPLAGTCGVLLLSLVITLYC

SEQ ID NO: 10 - protein, 41 aa, Artificial Sequence
  CD28 amino acid
RSKRSRLLHSDYMNMTPRRPGPTRKHYQPYAPPRDFAAYRS

SEQ ID NO: 11 - protein, 42 aa, Artificial Sequence
  4-1BB amino acid
KRGRKKLLYIFKQPFMRPVQTTQEEDGCSCRFPEEEEGGCEL

SEQ ID NO: 12 - protein, 113 aa, Artificial Sequence
  CD3zeta amino acid
RVKFSRSADAPAYQQGQNQLYNELNLGRREEYDVLDKRRGRDPEMGGKPQRRKNPQEGLYNELQKDKMAEAYSEIGMKGERRRGKGHDGLYQGLSTATKDTYDALHMQALPPR

SEQ ID NO: 13 - DNA, 17 bp, Artificial Sequence
  CPL F
accaccacaccagctcc

SEQ ID NO: 14 - DNA, 18 bp, Artificial Sequence
  CPL R
aggtctagcagcatgcag

SEQ ID NO: 15 - DNA, 36 bp, Artificial Sequence
  E1 F
catgctgctagacctgtttctgatgttccgagggac

SEQ ID NO: 16 - DNA, 41 bp, Artificial Sequence
  E1 R
agctggtgtggtggttgttcggtaattaatggaaattgggc